European Patent Application EP 4 389 908 A2, published June 26, 2024. Title: PROTEIN. Applicant: GlaxoSmithKline Biologicals s.a. The sequence listing filed with the application follows.

SEQUENCE LISTING (14 sequences)

SEQ ID NO: 1 - protein, 713 aa, Campylobacter jejuni
MLKKEYLKNPYLVLFAMIILAYVFSVFCRFYWVWWASEFNEYFFNNQLMIISNDGYAFAEGARDMIAGFHQPNDLSYYGSSLSALTYWLYKITPFSFESIILYMSTFLSSLVVIPTILLANEYKRPLMGFVAALLASIANSYYNRTMSGYYDTDMLVIVLPMFILFFMVRMILKKDFFSLIALPLFIGIYLWWYPSSYTLNVALIGLFLIYTLIFHRKEKIFYIAVILSSLTLSNIAWFYQSAIIVILFALFALEQKRLNFMIIGILGSATLIFLILSGGVDPILYQLKFYIFRSDESANLTQGFMYFNVNQTIQEVENVDLSEFMRRISGSEIVFLFSLFGFVWLLRKHKSMIMALPILVLGFLALKGGLRFTIYSVPVMALGFGFLLSEFKAIMVKKYSQLTSNVCIVFATILTLAPVFIHIYNYKAPTVFSQNEASLLNQLKNIANREDYVVTWWDYGYPVRYYSDVKTLVDGGKHLGKDNFFPSFALSKDEQAAANMARLSVEYTEKSFYAPQNDILKTDILQAMMKDYNQSNVDLFLASLSKPDFKIDTPKTRDIYLYMPARMSLIFSTVASFSFINLDTGVLDKPFTFSTAYPLDVKNGEIYLSNGVVLSDDFRSFKIGDNVVSVNSIVEINSIKQGEYKITPIDDKAQFYIFYLKDSAIPYAQFILMDKTMFNSAYVQMFFLGNYDKNLFDLVINSRDAKVFKLKI

SEQ ID NO: 2 - protein, 713 aa, Campylobacter jejuni
MLKKEYLKNPYLVLFAMIILAYVFSVFCRFYWVWWASEFNEYFFNNQLMIISNDGYAFAEGARDMIAGFHQPNDLSRYGSSLSALTYWLYKITPFSFESIILYMSTFLSSLVVIPTILLANEYKRPLMGFVAALLASIANSYYNRTMSGYYDTDMLVIVLPMFILFFMVRMILKKDFFSLIALPLFIGIYLWWYPSSYTLNVALIGLFLIYTLIFHRKEKIFYIAVILSSLTLSNIAWFYQSAIIVILFALFALEQKRLNFMIIGILGSATLIFLILSGGVDPILYQLKFYIFRSDESANLTQGFMYFNVVQTIQEVENVDLSEFMRRISGSEIVFLFSLFGFVWLLRKHKSMIMALPILVLGFLALKGGLRFTIYSVPVMALGFGFLLSEFKAIMVKKYSQLTSNVCIVFATILTLAPVFIHIYNYKAPTVFSQNEASLLNQLKNIANREDYVVTWWDYGYPVRYYSDVKTLVDGGKHLGKDNFFPSFALSKDEQAAANMARLSVEYTEKSFYAPQNDILKTDILQAMMKDYNQSNVDLFLASLSKPDFKIDTPKTRDIYLYMPARMSLIFSTVASFSFINLDTGVLDKPFTFSTAYPLDVKNGEIYLSNGVVLSDDFRSFKIGDNVVSVNSIVEINSIKQGEYKITPIDDKAQFYIFYLKDSAIPYAQFILMDKTMFNSAYVQMFFLGNYDKNLFDLVINSRDAKVFKLKI

SEQ ID NO: 3 - protein, 713 aa, Campylobacter jejuni
MLKKEYLKNPYLVLFAMIILAYVFSVFCRFYWVWWASEFNEYFFNNQLMIISNDGYRFAEGARDMIAGFHQPNDLSRYGSSLSALTYWLYKITPFSFESIILYMSTFLSSLVVIPTILLANEYKRPLMGFVAALLASIANSYYNRTMSGYYDTDMLVIVLPMFILFFMVRMILKKDFFSLIALPLFIGIYLWWYPSSYTLNVALIGLFLIYTLIFHRKEKIFYIAVILSSLTLSNIAWFYQSAIIVILFALFALEQKRLNFMIIGILGSATLIFLILSGGVDPILYQLKFYIFRSDESANLTQGFMYFNVVQTIQEVENVDLSEFMRRISGSEIVFLFSLFGFVWLLRKHKSMIMALPILVLGFLALKGGLRFTIYSVPVMALGFGFLLSEFKAIMVKKYSQLTSNVCIVFATILTLAPVFIHIYNYKAPTVFSQNEASLLNQLKNIANREDYVVTWWDYGYPVRYYSDVKTLVDGGKHLGKDNFFPSFALSKDEQAAANMARLSVEYTEKSFYAPQNDILKTDILQAMMKDYNQSNVDLFLASLSKPDFKIDTPKTRDIYLYMPARMSLIFSTVASFSFINLDTGVLDKPFTFSTAYPLDVKNGEIYLSNGVVLSDDFRSFKIGDNVVSVNSIVEINSIKQGEYKITPIDDKAQFYIFYLKDSAIPYAQFILMDKTMFNSAYVQMFFLGNYDKNLFDLVINSRDAKVFKLKI

SEQ ID NO: 4 - protein, 713 aa, Campylobacter jejuni
MLKKEYLKNPYLVLFAMIILAYVFSVFCRFYWVWWASEFNEYFFNNQLMIISNDGYRFAEGARDMIAGFHQPNDLSRYGSSLSALTYWLYKITPFSFESIILYMSTFLSSLVVIPTILLANEYKRPLMGFVAALLASIANSYYNRTMSGYYDTDMLVIVLPMFILFFMVRMILKKDFFSLIALPLFIGIYLWWYPSSYTLNVALIGLFLIYTLIFHRKEKIFYIAVILSSLTLSNIAWFYQSAIIVILFALFALEQKRLNFMIIGILGSATLIFLILSGGVDPILYQLKFYIFRSDESALPTQGFMYWNVVQTIQEVENVDLSEFMRRISGSEIVFLFSLFGFVWLLRKHKSMIMALPILVLGFLALKGGLRFTIYSVPVMALGFGFLLSEFKAIMVKKYSQLTSNVCIVFATILTLAPVFIHIYNYKAPTVFSQNEASLLNQLKNIANREDYVVTWWDYGWPVRYYSDVKTLVDGGKMLGKDNFFPSFALSKDEQAAANMARLSVEYTEKSFYAPQNDILKTDILQAMMKDYNQSNVDLFLASLSKPDFKIDTPKTRDIYLYMPARMSRIFSTVASFSFINLDTGVLDKPFTFSTAYPLDVKNGEIYLSNGVVLSDDFRSFKIGDNVVSVNSIVEINSIKQGEYKITPIDDKAQFYIFYLKDSAIPYAQFILMDKTMFNSAYVQMFFLGNYDKNLFDLVINSRDAKVFKLKI

SEQ ID NO: 5 - protein, 713 aa, Campylobacter jejuni
MLKKEYLKNPYLVLFAMIILAYVFSVFCRFYWVWWASEFNEYFFNNQLMIISNDGYRFAEGARDMIAGFHQPNDLSRYGSSLSALTYWLYKITPFSFESIILYMSTFLSSLVVIPTILLANEYKRPLMGFVAALLASIANSYYNRTMSGYYDTDMLVIVLPMFILFFMVRMILKKDFFSLIALPLFIGIYYWWYPSSYTLNVALIGLFLIYTLIFHRKEKIFYIAVILSSLTLSNIAWFYQSAIIVILFALFALEQKRLNFMIIGILGSATLIFLILSGGVDPILQQLKFYIFRLDESALPTQGFMYWNVVQTIQEVENVDLSEFMRRISGSEIVFLFSLFGFVWLLRKHKSMIMALPILVLGFLALKGGLRFTIYSVPVMSLGFGFLLSEFKAIMVKKYSQLTSNVCIVFATILTLAPVFIHIYNYKAPTVFSQNEASLLNQLKNIANREDYVVTWWDYGWPVRYYSDVKTLVDGGKMLGRDNFFPSFALSKDEQAAANMARLSVEYTEKSFYAPQNDILKRDILQAMMKDYNQSNVDLFLASLSKPDFKIDTPKTRDIYLYMPARMSRIFSTVASFSFINLDTGVLDKPFTFSTAYPLDVKNGEIYLSNGVVLSDDFRSFKIGDNVVSVNSIVEINSIKQGEYKITPIDDKAQFYIFYLKDSAIPYAQFILMDKTMFNSAYVQMFFLGNYDKNLFDLVINSRDAKVFKLKI

SEQ ID NO: 6 - protein, 713 aa, Campylobacter jejuni
MLKKEYLKNPYLVLFAMIILAYVFSVFCRFYWVWWASEFNEYFFNNQLMIISNDGYRFAEGARDMIAGFHQPNDLSRYGSSLSALTYWLYKITPFSFESIILYMSTFLSSLVVIPTILLANEYKRPLMGFVAALLASIANSYYNRTMSGYYDTDMLVIVLPMFILFFMVRMILKKDFFSLIALPLFIGIYYWWYPSSYTLNVALIGLFLIYTLIFHRKEKIFYIAVILSSLTLSNIAWFYQSAIIVILFALFALEQKRLNFMIIGILGSATLIFLILSGGVDPILQQLKFYIFRLDRSALPTQGFMYWNVVQTIQEVENVDLSEFMRRISGSEIVFLFSLFGFVWLLRKHKSMIMALPILVLGFLALKGGLRFTIYSVPVMSLGFGFLLSEFKAIMVKKYSQLTSNVCIVFATILTLAPVFIHIYNYKAPTVFSQNEASLLNQLKNIANREDYVVTWWDYGWPVRYYSDVKTLVDGGKMLGRDNFFPSFALSKDEQAAANMARLSVEYTEKSFYAPQNDILKRDILQAMMKDYNQSNVDLFLASLSKPDFKIDTPKTRDIYLYMPARMSRIFSTVASFSFINLDTGVLDKPFTFSTAYPLDVKNGEIYLSNGVVLSDDFRSFKIGDNVVSVNSIVEINSIKQGEYKITPIDDKAQFYIFYLKDSAIPYAQFILMDKTMFNSAYVQMFFLGNYDKNLFDLVINSRDAKVFKLKI

SEQ ID NO: 7 - protein, 713 aa, Campylobacter jejuni
MLKKEYLKNPYLVLFAMIILAYVFSVFCRFYWVWWASEFNEYFFNNQLMIISNDGYRFAEGARDMIAGFHQPNDLSRYGDSLSALTYWLYKITPFSFESIILYMSTFLSSLVVIPTILLANEYKRPLMGFVAALLASIANSYYNRTMSGYYDTDMLVIVLPMFILFFMVRMILKKDFFSLIALPLFIGIYYWWYPSSYTLNVALIGLFLIYTLIFHRKEKIFYIAVILSSLTLSNIAWFYQSAIIVILFALFALEQKRLNFMIIGILGSATLIFLILSGGVDPILQQLKFYIFRLDRSALPTQGFMYWNVVQTIQEVENVDLSEFMRRISGSEIVFLFSLFGFVWLLRKHKSMIMALPILVLGFLALKGGLRFTIYSVPVMSLGFGFLLSEFKAIMVKKYSQLTSNVCIVFATILTLAPVFIHIYNYKAPTVFSQNEASLLNQLKNIANREDYVVTWWDYGWPVRYYSDVKTLVDGGKMLGRDNFFPSFALSKDEQAAANMARLSVEYTEKSFYAPQNDILKRDILQAMMKDYNQSNVDLFLASLSKPDFKIDTPKTRDIYLYMPARMSRIFSTVASFSFINLDTGVLDKPFTFSTAYPLDVKNGEIYLSNGVVLSDDFRSFKIGDNVVSVNSIVEINSIKQGEYKITPIDDKAQFYIFYLKDSAIPYAQFILMDKTMFNSAYVQMFFLGNYDKNLFDLVINSRDAKVFKLKI

SEQ ID NO: 8 - protein, 713 aa, Campylobacter jejuni
MLKKEYLKNPYLVLFAMIILAYVFSVFCRFYWVWWASEFNEYFFNNQLMIISNDGYRFAEGARDMIAGFHQPNDLSRYGDSLSALTYWLYKITPFSFESIILYMSTFLSSLVVIPTILLANEYKRPLMGFVAALLASIANSYYNRTMSGYYDTDMLVIVLPMFILFFMVRMILKKDFFSLIALPLFVGIYYWWYPSSYTLNVALIGLFLIYTLIFHRKEKIFYIAVILSSLTLSNIAWFYQSAIIVILFALFALEQKRLNFMIIGILGSATLIFLILSGGVDPILQQLKFYIFRLDRSALPTQGFMYWNVVQTIQEVENVDLSEFMRRISGSEIVFLFSLFGFVWLLRKHKSMIMALPQLVLGFLALKGGLRFTIYSVPVMSLGFGFLLSEFKAIMVKKYSQLTSIVCIVFATILTLAPVFIHIYNYKAPTVFSQNEASLLNQLKNIANREDYVVTWWDYGWPVRYYSDVKTLVDGGKMLGRDNFFPSFALSKDEQAAANMARLSVEYTEKSFYAPQNDILKRDILQAMMKDYNQSNVDLFLASLSKPDFKIDTPKTRDIYLYMPARMSRIFSTVASFSFINLDTGVLDKPFTFSTAYPLDVKNGEIYLSNGVVLSDDFRSFKIGDNVVSVNSIVEINSIKQGEYKITPIDDKAQFYIFYLKDSAIPYAQFILMDKTMFNSAYVQMFFLGNYDKNLFDLVINSRDAKVFKLKI

SEQ ID NO: 9 - protein, 722 aa, Campylobacter jejuni
MLKKEYLKNPYLVLFAMIILAYVFSVFCRFYWVWWASEFNEYFFNNQLMIISNDGYAFAEGARDMIAGFHQPNDLSYYGSSLSALTYWLYKITPFSFESIILYMSTFLSSLVVIPTILLANEYKRPLMGFVAALLASIANSYYNRTMSGYYDTDMLVIVLPMFILFFMVRMILKKDFFSLIALPLFIGIYLWWYPSSYTLNVALIGLFLIYTLIFHRKEKIFYIAVILSSLTLSNIAWFYQSAIIVILFALFALEQKRLNFMIIGILGSATLIFLILSGGVDPILYQLKFYIFRSDESANLTQGFMYFNVNQTIQEVENVDLSEFMRRISGSEIVFLFSLFGFVWLLRKHKSMIMALPILVLGFLALKGGLRFTIYSVPVMALGFGFLLSEFKAIMVKKYSQLTSNVCIVFATILTLAPVFIHIYNYKAPTVFSQNEASLLNQLKNIANREDYVVTWWDYGYPVRYYSDVKTLVDGGKHLGKDNFFPSFALSKDEQAAANMARLSVEYTEKSFYAPQNDILKTDILQAMMKDYNQSNVDLFLASLSKPDFKIDTPKTRDIYLYMPARMSLIFSTVASFSFINLDTGVLDKPFTFSTAYPLDVKNGEIYLSNGVVLSDDFRSFKIGDNVVSVNSIVEINSIKQGEYKITPIDDKAQFYIFYLKDSAIPYAQFILMDKTMFNSAYVQMFFLGNYDKNLFDLVINSRDAKVFKLKIYPYDVPDYA

SEQ ID NO: 10 - protein, 712 aa, Campylobacter lari
MKLQQNFTDNNSIKYTCILILIAFAFSVLCRLYWVAWASEFYEFFFNDQLMITTNDGYAFAEGARDMIAGFHQPNDLSYFGSSLSTLTYWLYSILPFSFESIILYMSAFFASLIVVPIILIAREYKLTTYGFIAALLGSIANSYYNRTMSGYYDTDMLVLVLPMLILLTFIRLTINKDIFTLLLSPVFIMIYLWWYPSSYSLNFAMIGLFGLYTLVFHRKEKIFYLTIALMIIALSMLAWQYKLALIVLLFAIFAFKEEKINFYMIWALIFISILILHLSGGLDPVLYQLKFYVFKASDVQNLKDAAFMYFNVNETIMEVNTIDPEVFMQRISSSVLVFILSFIGFILLCKDHKSMLLALPMLALGFMALRAGLRFTIYAVPVMALGFGYFLYAFFNFLEKKQIKLSLRNKNILLILIAFFSISPALMHIYYYKSSTVFTSYEASILNDLKNKAQREDYVVAWWDYGYPIRYYSDVKTLIDGGKHLGKDNFFSSFVLSKEQIPAANMARLSVEYTEKSFKENYPDVLKAMVKDYNKTSAKDFLESLNDKDFKFDTNKTRDVYIYMPYRMLRIMPVVAQFANTNPDNGEQEKSLFFSQANAIAQDKTTGSVMLDNGVEIINDFRALKVEGASIPLKAFVDIESITNGKFYYNEIDSKAQIYLLFLREYKSFVILDESLYNSSYIQMFLLNQYDQDLFEQITNDTRAKIYRLKR

SEQ ID NO: 11 - protein, 713 aa, Campylobacter jejuni
MLKKEYLKNPYLVLFAMIILAYVFSVFCRFYWVWWASEFNEYFFNNQLMIISNDGYAFAEGARDMIAGFHQPNDLSHYGSSLSALTYWLYKITPFSFESIILYMSTFLSSLVVIPTILLANEYKRPLMGFVAALLASIANSYYNRTMSGYYDTDMLVIVLPMFILFFMVRMILKKDFFSLIALPLFIGIYLWWYPSSYTLNVALIGLFLIYTLIFHRKEKIFYIAVILSSLTLSNIAWFYQSAIIVILFALFALEQKRLNFMIIGILGSATLIFLILSGGVDPILYQLKFYIFRSDESANLTQGFMYFNVVQTIQEVENVDLSEFMRRISGSEIVFLFSLFGFVWLLRKHKSMIMALPILVLGFLALKGGLRFTIYSVPVMALGFGFLLSEFKAIMVKKYSQLTSNVCIVFATILTLAPVFIHIYNYKAPTVFSQNEASLLNQLKNIANREDYVVTWWDYGYPVRYYSDVKTLVDGGKHLGKDNFFPSFALSKDEQAAANMARLSVEYTEKSFYAPQNDILKTDILQAMMKDYNQSNVDLFLASLSKPDFKIDTPKTRDIYLYMPARMSLIFSTVASFSFINLDTGVLDKPFTFSTAYPLDVKNGEIYLSNGVVLSDDFRSFKIGDNVVSVNSIVEINSIKQGEYKITPIDDKAQFYIFYLKDSAIPYAQFILMDKTMFNSAYVQMFFLGNYDKNLFDLVINSRDAKVFKLKI

SEQ ID NO: 12 - protein, 714 aa, Campylobacter coli
MLKKEYFKNPTFILLAFIILAYVFSVLCRFYWIFWASEFNEYFFNNELMIISNDGYAFAEGARDMIAGFHQPNDLSYYGSSLSTLTYWFYKITPFSLESIFIYISTFLSSLVVIPLILIANEYKRPLMGFVAALLASIANSYYNRTMSGYYDTDMLVIVLAMMIVFFMIRLILKKDLLSLITLPLFVGIYLWWYPSSYTLNVALLGLFFIYTLVFHIKEKTLYMAIILASITLSNIAWFYQSAIIVILFSLFVLQNKRFSFALLGILGLATLVFLILSGGIDPILYQLKFYIFRSDESANLAQGFMYFNVNQTIQEVESIDLSIFMQRISGSELVFFVSLIGFIFLVRKHKSMILALPMLALGFLALKSGLRFTIYAVPVLALGFGFLMSLLQERKQKNNNTYWWANIGVFIFTFLSLIPMFYHINNYKAPTVFSQNEATKLDELKKIAQREDYVVTWWDYGYPIRYYSDVKTLADGGKHLGKDNFFPSFVLSKDQVAAANMARLSVEYTEKSFYAPLNDILKNDLLQAMMKDYNQNNVDLFLASLSKPDFKINMPKTRDVYIYMPARMSLIFSTVASFSFVDLETGEINKPFTFSAAYPLDVKNGEIYLSNGIALSDDFRSFKINNSTISVNSIIEINSIKQGEYKITPIDDMAQFYIFYLKDSTIPYAQFILMDKTMFNSAYVQMFFLGNYDKNLYDLVINARDAKVFKLKI

SEQ ID NO: 13 - protein, 711 aa, Campylobacter coli
MLKKEYFKNPTFILLTLIILAYAFSVLCRFYWVFWASEFNEYFFNNELMIISNDGYAFAEGARDMIAGFHQPNDLSYYGSSLSTLTYWFYKITPFSLESIFIYISTFLSSLVVVPLILIANEYKRPLMGFVAALLASIANSYYNRTMSGYYDTDMLVIVLAMMIVFFMIRLILRKDLLSLIALPLFVGIYLWWYPSSYTLNVALLGLLFIYTLVFHIKEKTLYMAIILASITLSNIAWFYQSAIIVILFSLFVLQNKRFSFALLGFLGLATLVFLILSGGVDPILYQLKFYIFRSDESANLAQGFMYFNVNQTIQEVESIDLSIFMKRISGSELVFFISLIGFIFLVRKHKSMILALPMLALGFLALKGGLRFTIYAVPVLALGFGFLMSLLQERKWKNKNIYWASVSIFTFLSLLPMFYHIINYKAPTVFSQNEASKLDELKKIAQREDYVVAWWDYGYPIRYYSDVKTLADGGKHLGKDNFFPSFILSKDQTAAANMARLSVEYTEKSFYAPSNDILKNDLLKAMMKDYKQNNVDLFLASLSKPDFKINTPKTRDVYIYMPARMSLIFSTVASFSFVDLDTGKIDKPFTFSAAYPLDVKNGEIYLSNGIVLSDDFRSFKINHNTIPVNSIIEVSSIKQGEYKITPIDDTAQFYILYLKDSTIPYAQFILMDKAMFNSAYVQMFFLGNYDKNLYDLVINTRDTKVFKLKI

SEQ ID NO: 14 - protein, 714 aa, Campylobacter coli
MLKKEYFKNPTFILLAFIILAYVFSVLCRFYWVFWASEFNEYFFNNELMIISNDGYAFAEGARDMIAGFHQPNDLSYYGSSLSTLTYWFYKITPFSLESIFIYISTFLSSLVVIPLILIANEYKRPLMGFVAALLASIANSYYNRTMSGYYDTDMLVIVLAMMIVFFMIRLILKKDLLSLIALPLFVGIYLWWYPSSYTLNVALLGLFFIYTLVFHIKEKTLYMAIILASITLSNIAWFYQSAIIVILFSLFVLQNKRFSFALLGILGLATLVFLILSGGIDPILYQLKFYIFRSDESANLAQGFMYFNVNQTIQEVESIDLSIFMQRISGSELVFFVSLIGFIFLVRKHKSMILALPMLALGFLALKSGLRFTIYAVPVLALGFGFLMSLLQERKQKNNNTYWWANIGVFIFTFLSLIPMFYHINNYKAPTVFSQNEATKLDELKKIAQREDYVVAWWDYGYPIRYYSDVKTLADGGKHLGKDNFFPSFVLSKDQVAAANMARLSVEYTEKSFYAPLNDILKNDLLQAMMKDYNQNNVDLFLALLSKPDFKINTPKTRDVYIYMPARMSLIFSTVASFSFVDLGTGEINKPFTFSAAYPLDVKNGEIYLSNGIVLSDDFRSFKINNSTISVNSIIEINSIKQGEYKITPIDDTAQFYIFYLKDSTIPYAQFILMDKTMFNSAYVQMFFLGNYDKNLYDLVINARDAKVFKLKF